European Patent Specification EP 4 075 980 B1, published July 23, 2025. Title: SUBSTITUTED 1,2,4-TRIAZOLES AND METHODS OF USE. Applicant: STINGINN LLC Glen, Barber N. The sequence listing filed with the application follows.

SEQUENCE LISTING (1 sequence)

SEQ ID NO: 1 - protein, 237 aa, Artificial Sequence
  Synthetic polypeptide
MNFNVAHGLAWSYYIGYLRLILPELQARIRTYNQHYNNLLRGAVSQRLYILLPLDCGVPDNLSMADPNIRFLDKLPQQTGDHAGIKDRVYSNSIYELLENGQRAGTCVLEYATPLQTLFAMSQYSQAGFSREDRLEQAKLFCRTLEDILADAPESQNNCRLIAYQEPADDSSFSLSQEVLRHLRQEEKEEVTVGSLKTSAVPSTSTMSQEPELLISGMEKPLPLRTDFSLEHHHHHH